European Patent Specification EP 3 752 633 B1, published November 29, 2023. Title: Verfahren und Vorrichtung zum Extrahieren einer Nukleinsäure aus einer Probenflüssigkeit. Applicant: GNA Biosolutions GmbH. The sequence listing filed with the application follows.

SEQUENCE LISTING (4 sequences)

SEQ ID NO: 1 - DNA, 23 bp, Artificial seqence
  synthetische funktionelle Nukleinsäure
tgaagatgtgcttacaagtgcta

SEQ ID NO: 2 - DNA, 24 bp, Artificial sequence
  synthetische funktionelle Nukleinsäure
tccaccctcaaacaggtgaattat

SEQ ID NO: 3 - DNA, 35 bp, Artificial sequence
  synthetische funktionelle Nukleinsäure
aaaaaaaaaaaaaaaaaaaaaaaaaaaaaaaaaaa

SEQ ID NO: 4 - DNA, 24 bp, Artificial Sequence
  synthetische funktionelle Nukleinsäure
aaatgattatggctcaggtactgc